European Patent Application EP 4 578 962 A1, published July 2, 2025. Title: Composition for amplifying FLT3 gene and Uses thereof. Applicant: NGeneBio. The sequence listing filed with the application follows.

SEQUENCE LISTING (36 sequences)

SEQ ID NO: 1 - DNA, 26 bp, synthetic construct
  source 1..26: mol_type = other DNA
cgtgcattttaaagattttccaatgg

SEQ ID NO: 2 - DNA, 24 bp, synthetic construct
  source 1..24: mol_type = other DNA
gaactgcctattcctaactgactc

SEQ ID NO: 3 - DNA, 24 bp, synthetic construct
  source 1..24: mol_type = other DNA
tgctgtccttccactatactgtac

SEQ ID NO: 4 - DNA, 24 bp, synthetic construct
  source 1..24: mol_type = other DNA
gccaaatgtttctgcagcatttct

SEQ ID NO: 5 - DNA, 20 bp, synthetic construct
  source 1..20: mol_type = other DNA
ggaaactgtgcctcccattt

SEQ ID NO: 6 - DNA, 23 bp, synthetic construct
  source 1..23: mol_type = other DNA
gcttttggaaaagtgatgaacgc

SEQ ID NO: 7 - DNA, 23 bp, synthetic construct
  source 1..23: mol_type = other DNA
cctgttttgctaattccataagc

SEQ ID NO: 8 - DNA, 22 bp, synthetic construct
  source 1..22: mol_type = other DNA
gatctcaaatgggagtttccaa

SEQ ID NO: 9 - DNA, 20 bp, synthetic construct
  source 1..20: mol_type = other DNA
ctgcagaaacatttggcaca

SEQ ID NO: 10 - DNA, 21 bp, synthetic construct
  source 1..21: mol_type = other DNA
gccagctacagatggtacagg

SEQ ID NO: 11 - DNA, 20 bp, synthetic construct
  source 1..20: mol_type = other DNA
tcattatctgaggagccggt

SEQ ID NO: 12 - DNA, 22 bp, synthetic construct
  source 1..22: mol_type = other DNA
cctcttcattgtcgttttaacc

SEQ ID NO: 13 - DNA, 23 bp, synthetic construct
  source 1..23: mol_type = other DNA
ggcactcatgtcagaactcaaga

SEQ ID NO: 14 - DNA, 23 bp, synthetic construct
  source 1..23: mol_type = other DNA
aggcattctttattttgacccct

SEQ ID NO: 15 - DNA, 22 bp, synthetic construct
  source 1..22: mol_type = other DNA
cagagaaccaagccctcctaag

SEQ ID NO: 16 - DNA, 22 bp, synthetic construct
  source 1..22: mol_type = other DNA
tggatgtgattggaaagtgggg

SEQ ID NO: 17 - DNA, 20 bp, synthetic construct
  source 1..20: mol_type = other DNA
ggcacagcccagtaaagata

SEQ ID NO: 18 - DNA, 20 bp, synthetic construct
  source 1..20: mol_type = other DNA
aaatagcagcctcacattgc

SEQ ID NO: 19 - DNA, 59 bp, synthetic construct
  source 1..59: mol_type = other DNA
tcgtcggcagcgtcagatgtgtataagagacagcgtgcattttaaagattttccaatgg

SEQ ID NO: 20 - DNA, 58 bp, synthetic construct
  source 1..58: mol_type = other DNA
gtctcgtgggctcggagatgtgtataagagacaggaactgcctattcctaactgactc

SEQ ID NO: 21 - DNA, 57 bp, synthetic construct
  source 1..57: mol_type = other DNA
tcgtcggcagcgtcagatgtgtataagagacagtgctgtccttccactatactgtac

SEQ ID NO: 22 - DNA, 58 bp, synthetic construct
  source 1..58: mol_type = other DNA
gtctcgtgggctcggagatgtgtataagagacaggccaaatgtttctgcagcatttct

SEQ ID NO: 23 - DNA, 53 bp, synthetic construct
  source 1..53: mol_type = other DNA
tcgtcggcagcgtcagatgtgtataagagacagggaaactgtgcctcccattt

SEQ ID NO: 24 - DNA, 57 bp, synthetic construct
  source 1..57: mol_type = other DNA
gtctcgtgggctcggagatgtgtataagagacaggcttttggaaaagtgatgaacgc

SEQ ID NO: 25 - DNA, 56 bp, synthetic construct
  source 1..56: mol_type = other DNA
tcgtcggcagcgtcagatgtgtataagagacagcctgttttgctaattccataagc

SEQ ID NO: 26 - DNA, 56 bp, synthetic construct
  source 1..56: mol_type = other DNA
gtctcgtgggctcggagatgtgtataagagacaggatctcaaatgggagtttccaa

SEQ ID NO: 27 - DNA, 53 bp, synthetic construct
  source 1..53: mol_type = other DNA
tcgtcggcagcgtcagatgtgtataagagacagctgcagaaacatttggcaca

SEQ ID NO: 28 - DNA, 55 bp, synthetic construct
  source 1..55: mol_type = other DNA
gtctcgtgggctcggagatgtgtataagagacaggccagctacagatggtacagg

SEQ ID NO: 29 - DNA, 53 bp, synthetic construct
  source 1..53: mol_type = other DNA
tcgtcggcagcgtcagatgtgtataagagacagtcattatctgaggagccggt

SEQ ID NO: 30 - DNA, 56 bp, synthetic construct
  source 1..56: mol_type = other DNA
gtctcgtgggctcggagatgtgtataagagacagcctcttcattgtcgttttaacc

SEQ ID NO: 31 - DNA, 56 bp, synthetic construct
  source 1..56: mol_type = other DNA
tcgtcggcagcgtcagatgtgtataagagacagggcactcatgtcagaactcaaga

SEQ ID NO: 32 - DNA, 57 bp, synthetic construct
  source 1..57: mol_type = other DNA
gtctcgtgggctcggagatgtgtataagagacagaggcattctttattttgacccct

SEQ ID NO: 33 - DNA, 55 bp, synthetic construct
  source 1..55: mol_type = other DNA
tcgtcggcagcgtcagatgtgtataagagacagcagagaaccaagccctcctaag

SEQ ID NO: 34 - DNA, 56 bp, synthetic construct
  source 1..56: mol_type = other DNA
gtctcgtgggctcggagatgtgtataagagacagtggatgtgattggaaagtgggg

SEQ ID NO: 35 - DNA, 53 bp, synthetic construct
  source 1..53: mol_type = other DNA
tcgtcggcagcgtcagatgtgtataagagacagggcacagcccagtaaagata

SEQ ID NO: 36 - DNA, 54 bp, synthetic construct
  source 1..54: mol_type = other DNA
gtctcgtgggctcggagatgtgtataagagacagaaatagcagcctcacattgc